European Patent Application EP 4 201 955 A1, published June 28, 2023. Title: T-CELL RECEPTORS DIRECTED AGAINST THE PREFERENTIALLY EXPRESSED ANTIGEN OF MELANOMA AND USES THEREOF. Applicant: Academisch Ziekenhuis Leiden H.O.D.N. Leids Universitair Medisch Centrum. Application EP. The sequence listing filed with the application follows.

SEQUENCE LISTING (108 sequences)

SEQ ID NO: 1 - protein, 24 aa, synthetic construct
  REGION 1..24: note = a CDR3 AA
CAVSGQTGANNLFFGTGTRLTVIP

SEQ ID NO: 2 - DNA, 72 bp, synthetic construct
  source 1..72: mol_type = other DNA
  misc_feature 1..72: note = a CDR3 NT
tgtgctgtgagtggccaaactggggcaaacaacctcttctttgggactggaacgagactcaccgttattccc

SEQ ID NO: 3 - DNA, 72 bp, synthetic construct
  source 1..72: mol_type = other DNA
  misc_feature 1..72: note = a CDR3 NT co*
tgtgccgtgagcggccagaccggcgccaacaacctgttcttcggcaccggcacccggctgacagtgatccct

SEQ ID NO: 4 - protein, 23 aa, synthetic construct
  REGION 1..23: note = B CDR3 AA
CASARWDRGGEQYFGPGTRLTVT

SEQ ID NO: 5 - DNA, 69 bp, synthetic construct
  source 1..69: mol_type = other DNA
  misc_feature 1..69: note = b CDR3 NT
tgtgccagcgcgaggtgggacaggggaggcgagcagtacttcgggccgggcaccaggctcacggtcaca

SEQ ID NO: 6 - DNA, 69 bp, synthetic construct
  source 1..69: mol_type = other DNA
  misc_feature 1..69: note = b CDR3 NT co
tgcgccagcgccagatgggatagaggcggcgagcagtacttcggccctggcaccagactgaccgtgacc

SEQ ID NO: 7 - protein, 133 aa, synthetic construct
  REGION 1..133: note = a VJ AA
MLLLLVPVLEVIFTLGGTRAQSVTQLGSHVSVSERALVLLRCNYSSSVPPYLFWYVQYPNQGLQLLLKYTSAATLVKGINGFEAEFKKSETSFHLTKPSAHMSDAAEYFCAVSGQTGANNLFFGTGTRLTVIP

SEQ ID NO: 8 - DNA, 399 bp, synthetic construct
  source 1..399: mol_type = other DNA
  misc_feature 1..399: note = a VJ NT
atgctcctgctgctcgtcccagtgctcgaggtgatttttaccctgggaggaaccagagcccagtcggtgacccagcttggcagccacgtctctgtctctgaacgagccctggttctgctgaggtgcaactactcatcgtctgttccaccatatctcttctggtatgtgcaataccccaaccaaggactccagcttctcctgaagtacacatcagcggccaccctggttaaaggcatcaacggttttgaggctgaatttaagaagagtgaaacctccttccacctgacgaaaccctcagcccatatgagcgacgcggctgagtacttctgtgctgtgagtggccaaactggggcaaacaacctcttctttgggactggaacgagactcaccgttattccc

SEQ ID NO: 9 - DNA, 399 bp, synthetic construct
  source 1..399: mol_type = other DNA
  misc_feature 1..399: note = a VJ NT co
atgctgctgctgctggtgcccgtgctggaagtgatcttcaccctgggcggcaccagagcccagagcgtgacacagctgggcagccacgtgtccgtgtctgagagggccctggtgctgctgagatgcaactactcttctagcgtgcccccctacctgttttggtacgtgcagtaccccaaccaggggctgcagctgctcctgaagtacaccagcgccgccacactggtgaagggcatcaacggcttcgaggccgagttcaagaagtccgagacaagcttccacctgaccaagcccagcgcccacatgtctgacgccgccgagtacttctgtgccgtgagcggccagaccggcgccaacaacctgttcttcggcaccggcacccggctgacagtgatccct

SEQ ID NO: 10 - protein, 123 aa, synthetic construct
  REGION 1..123: note = b VDJ AA
MGFRLLCCVAFCLLGAGPVDSGVTQTPKHLITATGQRVTLRCSPRSGDLSVYWYQQSLDQGLQFLIQYYNGEERAKGNILERFSAQQFPDLHSELNLSSLELGDSALYFCASARWDRGGEQYF

SEQ ID NO: 11 - DNA, 396 bp, synthetic construct
  source 1..396: mol_type = other DNA
  misc_feature 1..396: note = b VDJ NT
atgggcttcaggctcctctgctgtgtggccttttgtctcctgggagcaggcccagtggattctggagtcacacaaaccccaaagcacctgatcacagcaactggacagcgagtgacgctgagatgctcccctaggtctggagacctctctgtgtactggtaccaacagagcctggaccagggcctccagttcctcattcagtattataatggagaagagagagcaaaaggaaacattcttgaacgattctccgcacaacagttccctgacttgcactctgaactaaacctgagctctctggagctgggggactcagctttgtatttctgtgccagcgcgaggtgggacaggggaggcgagcagtacttcgggccgggcaccaggctcacggtcaca

SEQ ID NO: 12 - DNA, 396 bp, synthetic construct
  source 1..396: mol_type = other DNA
  misc_feature 1..396: note = b VDJ NT co
atgggcttccggctgctgtgctgcgtggccttttgtctgctgggagccggccctgtggatagcggcgtgacccagacccccaagcacctgatcaccgccaccggccagagagtgaccctgcgctgcagccctagaagcggcgacctgagcgtgtactggtatcagcagagcctcgaccagggcctgcagttcctgatccagtactacaacggcgaggaacgggccaagggcaacatcctggaacggttcagcgcccagcagttccccgatctgcacagcgagctgaacctgagcagcctggaactgggcgacagcgccctgtacttctgcgccagcgccagatgggatagaggcggcgagcagtacttcggccctggcaccagactgaccgtgacc

SEQ ID NO: 13 - protein, 274 aa, synthetic construct
  REGION 1..274: note = a VJ and constant AA
MLLLLVPVLEVIFTLGGTRAQSVTQLGSHVSVSERALVLLRCNYSSSVPPYLFWYVQYPNQGLQLLLKYTSAATLVKGINGFEAEFKKSETSFHLTKPSAHMSDAAEYFCAVSGQTGANNLFFGTGTRLTVIPYIQNPDPAVYQLRDSKSSDKSVCLFTDFDSQTNVSQSKDSDVYITDKCVLDMRSMDFKSNSAVAWSNKSDFACANAFNNSIIPEDTFFPSPESSCDVKLVEKSFETDTNLNFQNLSVIGFRILLLKVAGFNLLMTLRLWSS

SEQ ID NO: 14 - protein, 270 aa
MLLLLVPVLEVIFTLGGTRAQSVTQLGSHVSVSERALVLLRCNYSSSVPPYLFWYVQYPNQGLQLLLKYTSAATLVKGINGFEAEFKKSETSFHLTKPSAHMSDAAEYFCAVSGQTGANNLFFGTGTRLTVIPDIQNPEPAVYQLKDPRSQDSTLCLFTDFDSQINVPKTMESGTFITDKCVLDMKAMDSKSNGAIAWSNQTSFTCQDIFKETNATYPSSDVPCDATLTEKSFETDMNLNFQNLSVMGLRILLLKVAGFNLLMTLRLWSS

SEQ ID NO: 15 - DNA, 825 bp, synthetic construct
  source 1..825: mol_type = other DNA
  misc_feature 1..825: note = a VJ and constant NT
atgctcctgctgctcgtcccagtgctcgaggtgatttttaccctgggaggaaccagagcccagtcggtgacccagcttggcagccacgtctctgtctctgaacgagccctggttctgctgaggtgcaactactcatcgtctgttccaccatatctcttctggtatgtgcaataccccaaccaaggactccagcttctcctgaagtacacatcagcggccaccctggttaaaggcatcaacggttttgaggctgaatttaagaagagtgaaacctccttccacctgacgaaaccctcagcccatatgagcgacgcggctgagtacttctgtgctgtgagtggccaaactggggcaaacaacctcttctttgggactggaacgagactcaccgttattccctatatccagaaccctgaccctgccgtgtaccagctgagagactctaaatccagtgacaagtctgtctgcctattcaccgattttgattctcaaacaaatgtgtcacaaagtaaggattctgatgtgtatatcacagacaaatgcgtgctagacatgaggtctatggacttcaagagcaacagtgctgtggcctggagcaacaaatctgactttgcatgtgcaaacgccttcaacaacagcattattccagaagacaccttcttccccagcccagaaagttcctgtgatgtcaagctggtcgagaaaagctttgaaacagatacgaacctaaactttcaaaacctgtcagtgattgggttccgaatcctcctcctgaaagtggccgggtttaatctgctcatgacgctgcggttgtggtccagctga

SEQ ID NO: 16 - DNA, 825 bp, synthetic construct
  source 1..825: mol_type = other DNA
  misc_feature 1..825: note = a VJ and constant NT co
atgctgctgctgctggtgcccgtgctggaagtgatcttcaccctgggcggcaccagagcccagagcgtgacacagctgggcagccacgtgtccgtgtctgagagggccctggtgctgctgagatgcaactactcttctagcgtgcccccctacctgttttggtacgtgcagtaccccaaccaggggctgcagctgctcctgaagtacaccagcgccgccacactggtgaagggcatcaacggcttcgaggccgagttcaagaagtccgagacaagcttccacctgaccaagcccagcgcccacatgtctgacgccgccgagtacttctgtgccgtgagcggccagaccggcgccaacaacctgttcttcggcaccggcacccggctgacagtgatcccttacatccagaaccccgaccccgccgtgtaccagctgcgggacagcaagagcagcgacaagagcgtgtgcctgttcaccgacttcgacagccagaccaacgtgtcccagagcaaggacagcgacgtgtacatcaccgataagtgcgtgctggacatgcggagcatggacttcaagagcaacagcgccgtggcctggtccaacaagagcgacttcgcctgcgccaacgccttcaacaacagcatcatccccgaggacacattcttcccaagccccgagagcagctgcgacgtgaagctggtggagaagtccttcgagacagacaccaacctgaacttccagaacctgtccgtgatcggcttcagaatcctgctgctgaaagtggccggcttcaacctgctgatgaccctgcggctgtggagcagctga

SEQ ID NO: 17 - skipped

SEQ ID NO: 18 - DNA, 813 bp, synthetic construct
  source 1..813: mol_type = other DNA
  misc_feature 1..813: note = a VJ and constant (murine) NT co
atgctgctgctgctggtgcccgtgctggaagtgatcttcaccctgggcggcaccagagcccagagcgtgacacagctgggcagccacgtgtccgtgtctgagagggccctggtgctgctgagatgcaactactcttctagcgtgcccccctacctgttttggtacgtgcagtaccccaaccaggggctgcagctgctcctgaagtacaccagcgccgccacactggtgaagggcatcaacggcttcgaggccgagttcaagaagtccgagacaagcttccacctgaccaagcccagcgcccacatgtctgacgccgccgagtacttctgtgccgtgagcggccagaccggcgccaacaacctgttcttcggcaccggcacccggctgacagtgatccctgacattcagaacccggaaccggctgtataccagctgaaggacccccgatctcaggatagtactctgtgcctgttcaccgactttgatagtcagatcaatgtgcctaaaaccatggaatccggaacttttattaccgacaagtgcgtgctggatatgaaagccatggacagtaagtcaaacggcgccatcgcttggagcaatcagacatccttcacttgccaggatatcttcaaggagaccaacgcaacatacccatcctctgacgtgccctgtgatgccaccctgacagagaagtctttcgaaacagacatgaacctgaattttcagaatctgagcgtgatgggcctgagaatcctgctgctgaaggtcgctgggtttaatctgctgatgacactgcggctgtggtcctcatga

SEQ ID NO: 19 - protein, 311 aa, synthetic construct
  REGION 1..311: note = b VJ and constant AA
MGFRLLCCVAFCLLGAGPVDSGVTQTPKHLITATGQRVTLRCSPRSGDLSVYWYQQSLDQGLQFLIQYYNGEERAKGNILERFSAQQFPDLHSELNLSSLELGDSALYFCASARWDRGGEQYFGPGTRLTVTEDLKNVFPPEVAVFEPSEAEISHTQKATLVCLATGFYPDHVELSVWWNGKEVHSGVCTDPQPLKEQPALNDSRYCLSSRLRVSATFWQNPRNHFRCQVQFYGLSENDEWTQDRAKPVTQIVSAEAWGRADCGFTSESYQQGVLSATILYEILLGKATLYAVLVSALVLMAMVKRKDSRG

SEQ ID NO: 20 - protein, 305 aa, synthetic construct
  REGION 1..305: note = beta VJ and constant (murine) AA
MGFRLLCCVAFCLLGAGPVDSGVTQTPKHLITATGQRVTLRCSPRSGDLSVYWYQQSLDQGLQFLIQYYNGEERAKGNILERFSAQQFPDLHSELNLSSLELGDSALYFCASARWDRGGEQYFGPGTRLTVTEDLRNVTPPKVSLFEPSKAEIANKQKATLVCLARGFFPDHVELSVWWNGKEVHSGVCTDPQAYKESNYSYCLSSRLRVSATFWHNPRNHFRCQVQFHGLSEEDKWPEGSPKPVTQNISAEAWGRADCGITSASYHQGVLSATILYEILLGKATLYAVLVSGLVLMAMVKKKNS

SEQ ID NO: 21 - DNA, 933 bp, synthetic construct
  source 1..933: mol_type = other DNA
  misc_feature 1..933: note = b VJ and constant NT
atgggcttcaggctcctctgctgtgtggccttttgtctcctgggagcaggcccagtggattctggagtcacacaaaccccaaagcacctgatcacagcaactggacagcgagtgacgctgagatgctcccctaggtctggagacctctctgtgtactggtaccaacagagcctggaccagggcctccagttcctcattcagtattataatggagaagagagagcaaaaggaaacattcttgaacgattctccgcacaacagttccctgacttgcactctgaactaaacctgagctctctggagctgggggactcagctttgtatttctgtgccagcgcgaggtgggacaggggaggcgagcagtacttcgggccgggcaccaggctcacggtcacagaggacctgaaaaacgtgttcccacccgaggtcgctgtgtttgagccatcagaagcagagatctcccacacccaaaaggccacactggtgtgcctggccacaggcttctaccccgaccacgtggagctgagctggtgggtgaatgggaaggaggtgcacagtggggtctgcacagacccgcagcccctcaaggagcagcccgccctcaatgactccagatactgcctgagcagccgcctgagggtctcggccaccttctggcagaacccccgcaaccacttccgctgtcaagtccagttctacgggctctcggagaatgacgagtggacccaggatagggccaaacctgtcacccagatcgtcagcgccgaggcctggggtagagcagactgtggcttcacctccgagtcttaccagcaaggggtcctgtctgccaccatcctctatgagatcttgctagggaaggccaccttgtatgccgtgctggtcagtgccctcgtgctgatggccatggtcaagagaaaggattccagaggc

SEQ ID NO: 22 - DNA, 933 bp, synthetic construct
  source 1..933: mol_type = other DNA
  misc_feature 1..933: note = b VJ and constant NT co
atgggcttccggctgctgtgctgcgtggccttttgtctgctgggagccggccctgtggatagcggcgtgacccagacccccaagcacctgatcaccgccaccggccagagagtgaccctgcgctgcagccctagaagcggcgacctgagcgtgtactggtatcagcagagcctcgaccagggcctgcagttcctgatccagtactacaacggcgaggaacgggccaagggcaacatcctggaacggttcagcgcccagcagttccccgatctgcacagcgagctgaacctgagcagcctggaactgggcgacagcgccctgtacttctgcgccagcgccagatgggatagaggcggcgagcagtacttcggccctggcaccagactgaccgtgaccgaggacctgaagaacgtgttccccccagaggtggccgtgtttgagcccagcgaggccgagatcagccacacccagaaagccaccctggtgtgcctggccaccggcttctaccccgaccacgtggagctgtcttggtgggtgaacggcaaagaggtgcacagcggcgtctgcaccgacccccagcccctgaaagagcagcccgccctgaacgacagccggtactgcctgagcagcagactgcgggtgtccgccaccttctggcagaacccccggaaccacttccggtgccaggtgcagttctacggcctgagcgagaacgacgagtggacccaggacagagccaagcctgtgacccagatcgtgtctgccgaagcctggggcagagccgactgcggcttcaccagcgagagctaccagcagggcgtgctgagcgccaccatcctgtacgagatcctgctgggcaaggccacactgtacgccgtgctggtgtccgctctggtgctgatggccatggtgaagcggaaggacagcagaggc

SEQ ID NO: 23 - skipped

SEQ ID NO: 24 - DNA, 915 bp, synthetic construct
  source 1..915: mol_type = other DNA
  misc_feature 1..915: note = b VJ and constant (murine) NT co
atgggcttccggctgctgtgctgcgtggccttttgtctgctgggagccggccctgtggatagcggcgtgacccagacccccaagcacctgatcaccgccaccggccagagagtgaccctgcgctgcagccctagaagcggcgacctgagcgtgtactggtatcagcagagcctcgaccagggcctgcagttcctgatccagtactacaacggcgaggaacgggccaagggcaacatcctggaacggttcagcgcccagcagttccccgatctgcacagcgagctgaacctgagcagcctggaactgggcgacagcgccctgtacttctgcgccagcgccagatgggatagaggcggcgagcagtacttcggccctggcaccagactgaccgtgaccgaagatctacgtaacgtgacaccacccaaagtctcactgtttgagcctagcaaggcagaaattgccaacaagcagaaggccaccctggtgtgcctggcaagagggttctttccagatcacgtggagctgtcctggtgggtcaacggcaaagaagtgcattctggggtctgcaccgacccccaggcttacaaggagagtaattactcatattgtctgtcaagccggctgagagtgtccgccacattctggcacaaccctaggaatcatttccgctgccaggtccagtttcacggcctgagtgaggaagataaatggccagaggggtcacctaagccagtgacacagaacatcagcgcagaagcctggggacgagcagactgtggcattactagcgcctcctatcatcagggcgtgctgagcgccactatcctgtacgagattctgctgggaaaggccaccctgtatgctgtgctggtctccggcctggtgctgatggccatggtcaagaaaaagaactct

SEQ ID NO: 25 - protein, 25 aa, synthetic construct
  REGION 1..25: note = a CDR3 AA
CAGIPRDNYGQNFVFGPGTRLSVLP

SEQ ID NO: 26 - DNA, 75 bp, synthetic construct
  source 1..75: mol_type = other DNA
  misc_feature 1..75: note = a CDR3 NT
tgtgctgggataccccgggataactatggtcagaattttgtctttggtcccggaaccagattgtccgtgctgccc

SEQ ID NO: 27 - DNA, 75 bp, synthetic construct
  source 1..75: mol_type = other DNA
  misc_feature 1..75: note = a CDR3 NT co*
tgcgccggcatccctcgggacaactacggccagaacttcgtgttcggccctggcaccagactgagcgtgctgccc

SEQ ID NO: 28 - protein, 24 aa, synthetic construct
  REGION 1..24: note = beta CDR3 AA
CASTPWLAGGNEQFFGPGTRLTVL

SEQ ID NO: 29 - DNA, 72 bp, synthetic construct
  source 1..72: mol_type = other DNA
  misc_feature 1..72: note = b CDR3 NT
tgtgccagcaccccgtggctagcgggaggcaatgagcagttcttcgggccagggacacggctcaccgtgcta

SEQ ID NO: 30 - DNA, 72 bp, synthetic construct
  source 1..72: mol_type = other DNA
  misc_feature 1..72: note = b CDR3 NT co
tgtgccagcaccccttggctggctggcggcaacgagcagttttttggccctggcacccggctgaccgtgctg

SEQ ID NO: 31 - protein, 131 aa, synthetic construct
  REGION 1..131: note = a VJ AA
MLLEHLLIILWMQLTVWSGQQLNQSPQSMFIQEGEDVSMNCTSSSIFNTWLWYKQDPGEGPVLLIALYKAGELTSNGRLTAQFGITRKDSFLNISASIPSDVGIYFCAGIPRDNYGQNFVFGPGTRLSVLP

SEQ ID NO: 32 - DNA, 393 bp, synthetic construct
  source 1..393: mol_type = other DNA
  misc_feature 1..393: note = a VJ NT
atgctccttgaacatttattaataatcttgtggatgcagctgacatgggtcagtggtcaacagctgaatcagagtcctcaatctatgtttatccaggaaggagaagatgtctccatgaactgcacttcttcaagcatatttaacacctggctatggtacaagcaggaccctggggaaggtcctgtcctcttgatagccttatataaggctggtgaattgacctcaaatggaagactgactgctcagtttggtataaccagaaaggacagcttcctgaatatctcagcatccatacctagtgatgtaggcatctacttctgtgctgggataccccgggataactatggtcagaattttgtctttggtcccggaaccagattgtccgtgctgccc

SEQ ID NO: 33 - DNA, 393 bp, synthetic construct
  source 1..393: mol_type = other DNA
  misc_feature 1..393: note = a VJ NT co
atgctgctggaacatctgctgatcatcctgtggatgcagctgacctgggtgtccggccagcagctgaatcagagcccccagagcatgttcatccaggaaggcgaggacgtgtccatgaactgcaccagcagcagcatcttcaacacctggctgtggtacaagcaggaccccggcgaaggacccgtgctgctgatcgccctgtataaggccggcgagctgaccagcaacggcagactgacagcccagttcggcattacccggaaggacagcttcctgaacatcagcgccagcatccccagcgacgtgggcatctacttttgcgccggcatccctcgggacaactacggccagaacttcgtgttcggccctggcaccagactgagcgtgctgccc

SEQ ID NO: 34 - protein, 133 aa, synthetic construct
  REGION 1..133: note = B VDJ AA
MGIRLLCRVAFCFLAVGLVDVKVTQSSRYLVKRTGEKVFLECVQDMDHENMFWYRQDPGLGLRLIYFSYDVKMKEKGDIPEGYSVSREKKERFSLILESASTNQTSMYLCASTPWLAGGNEQFFGPGTRLTVL

SEQ ID NO: 35 - DNA, 399 bp, synthetic construct
  source 1..399: mol_type = other DNA
  misc_feature 1..399: note = b VDJ NT
atgggaatcaggctcctctgtcgtgtggccttttgtttcctggctgtaggcctcgtagatgtgaaagtaacccagagctcgagatatctagtcaaaaggacgggagagaaagtttttctggaatgtgtccaggatatggaccatgaaaatatgttctggtatcgacaagacccaggtctggggctacggctgatctatttctcatatgatgttaaaatgaaagaaaaaggagatattcctgaggggtacagtgtctctagagagaagaaggagcgcttctccctgattctggagtccgccagcaccaaccagacatctatgtacctctgtgccagcaccccgtggctagcgggaggcaatgagcagttcttcgggccagggacacggctcaccgtgcta

SEQ ID NO: 36 - DNA, 399 bp, synthetic construct
  source 1..399: mol_type = other DNA
  misc_feature 1..399: note = b VDJ NT co
atgggcatccggctgctgtgcagagtggccttctgctttctggccgtgggcctggtggacgtgaaagtgacccagagcagcagatacctcgtgaagcggaccggcgagaaggtgttcctggaatgcgtgcaggacatggaccacgagaatatgttctggtacagacaggaccccggcctgggcctgcggctgatctacttcagctacgacgtgaagatgaaggaaaagggcgacatccccgagggctacagcgtgtccagagagaagaaagagcggttcagcctgatcctggaaagcgccagcaccaaccagaccagcatgtacctgtgtgccagcaccccttggctggctggcggcaacgagcagttttttggccctggcacccggctgaccgtgctg

SEQ ID NO: 37 - protein, 272 aa, synthetic construct
  REGION 1..272: note = a VJ and constant AA
MLLEHLLIILWMQLTVWSGQQLNQSPQSMFIQEGEDVSMNCTSSSIFNTWLWYKQDPGEGPVLLIALYKAGELTSNGRLTAQFGITRKDSFLNISASIPSDVGIYFCAGIPRDNYGQNFVFGPGTRLSVLPYIQNPDPAVYQLRDSKSSDKSVCLFTDFDSQTNVSQSKDSDVYITDKTVLDMRSMDFKSNSAVAWSNKSDFACANAFNNSIIPEDTFFPSPESSCDVKLVEKSFETDTNLNFQNLSVIGFRILLLKVAGFNLLMTLRLWSS

SEQ ID NO: 38 - protein, 268 aa, synthetic construct
  REGION 1..268: note = a VJ and constant (murine) AA
MLLEHLLIILWMQLTVWSGQQLNQSPQSMFIQEGEDVSMNCTSSSIFNTWLWYKQDPGEGPVLLIALYKAGELTSNGRLTAQFGITRKDSFLNISASIPSDVGIYFCAGIPRDNYGQNFVFGPGTRLSVLPDIQNPEPAVYQLKDPRSQDSTLCLFTDFDSQINVPKTMESGTFITDKCVLDMKAMDSKSNGAIAWSNQTSFTCQDIFKETNATYPSSDVPCDATLTEKSFETDMNLNFQNLSVMGLRILLLKVAGFNLLMTLRLWSS

SEQ ID NO: 39 - protein, 819 aa, synthetic construct
  REGION 1..819: note = a VJ and constant NT
ATGCTCCTTGAACATTTATTAATAATCTTGTGGATGCAGCTGACATGGGTCAGTGGTCAACAGCTGAATCAGAGTCCTCAATCTATGTTTATCCAGGAAGGAGAAGATGTCTCCATGAACTGCACTTCTTCAAGCATATTTAACACCTGGCTATGGTACAAGCAGGACCCTGGGGAAGGTCCTGTCCTCTTGATAGCCTTATATAAGGCTGGTGAATTGACCTCAAATGGAAGACTGACTGCTCAGTTTGGTATAACCAGAAAGGACAGCTTCCTGAATATCTCAGCATCCATACCTAGTGATGTAGGCATCTACTTCTGTGCTGGGATACCCCGGGATAACTATGGTCAGAATTTTGTCTTTGGTCCCGGAACCAGATTGTCCGTGCTGCCCTATATCCAGAACCCTGACCCTGCCGTGTACCAGCTGAGAGACTCTAAATCCAGTGACAAGTCTGTCTGCCTATTCACCGATTTTGATTCTCAAACAAATGTGTCACAAAGTAAGGATTCTGATGTGTATATCACAGACAAAACTGTGCTAGACATGAGGTCTATGGACTTCAAGAGCAACAGTGCTGTGGCCTGGAGCAACAAATCTGACTTTGCATGTGCAAACGCCTTCAACAACAGCATTATTCCAGAAGACACCTTCTTCCCCAGCCCAGAAAGTTCCTGTGATGTCAAGCTGGTCGAGAAAAGCTTTGAAACAGATACGAACCTAAACTTTCAAAACCTGTCAGTGATTGGGTTCCGAATCCTCCTCCTGAAAGTGGCCGGGTTTAATCTGCTCATGACGCTGCGGTTGTGGTCCAGCTGA

SEQ ID NO: 40 - DNA, 819 bp, synthetic construct
  source 1..819: mol_type = other DNA
  misc_feature 1..819: note = a VJ and constant NT co
atgctgctggaacatctgctgatcatcctgtggatgcagctgacctgggtgtccggccagcagctgaatcagagcccccagagcatgttcatccaggaaggcgaggacgtgtccatgaactgcaccagcagcagcatcttcaacacctggctgtggtacaagcaggaccccggcgaaggacccgtgctgctgatcgccctgtataaggccggcgagctgaccagcaacggcagactgacagcccagttcggcattacccggaaggacagcttcctgaacatcagcgccagcatccccagcgacgtgggcatctacttttgcgccggcatccctcgggacaactacggccagaacttcgtgttcggccctggcaccagactgagcgtgctgccctacatccagaaccccgaccctgccgtgtaccagctgagagacagcaagagcagcgacaagagcgtgtgcctgttcaccgacttcgacagccagaccaacgtgtcccagagcaaggactccgacgtgtacatcaccgacaagaccgtgctggacatgcggagcatggacttcaagagcaacagcgccgtggcctggtccaacaagagcgatttcgcctgcgccaacgccttcaacaacagcattatccccgaggacacattcttcccaagccccgagagcagctgcgacgtgaagctggtggaaaagagcttcgagacagacaccaacctgaacttccagaacctgagcgtgatcggcttccggatcctgctgctgaaggtggccggcttcaacctgctgatgaccctgagactgtggtccagctga

SEQ ID NO: 41 - skipped

SEQ ID NO: 42 - DNA, 807 bp, synthetic construct
  source 1..807: mol_type = other DNA
  misc_feature 1..807: note = a VJ and constant (murine) NT co
atgctgctggaacatctgctgatcatcctgtggatgcagctgacctgggtgtccggccagcagctgaatcagagcccccagagcatgttcatccaggaaggcgaggacgtgtccatgaactgcaccagcagcagcatcttcaacacctggctgtggtacaagcaggaccccggcgaaggacccgtgctgctgatcgccctgtataaggccggcgagctgaccagcaacggcagactgacagcccagttcggcattacccggaaggacagcttcctgaacatcagcgccagcatccccagcgacgtgggcatctacttttgcgccggcatccctcgggacaactacggccagaacttcgtgttcggccctggcaccagactgagcgtgctgcccgacattcagaacccggaaccggctgtataccagctgaaggacccccgatctcaggatagtactctgtgcctgttcaccgactttgatagtcagatcaatgtgcctaaaaccatggaatccggaacttttattaccgacaagtgcgtgctggatatgaaagccatggacagtaagtcaaacggcgccatcgcttggagcaatcagacatccttcacttgccaggatatcttcaaggagaccaacgcaacatacccatcctctgacgtgccctgtgatgccaccctgacagagaagtctttcgaaacagacatgaacctgaattttcagaatctgagcgtgatgggcctgagaatcctgctgctgaaggtcgctgggtttaatctgctgatgacactgcggctgtggtcctcatga

SEQ ID NO: 43 - protein, 312 aa, synthetic construct
  REGION 1..312: note = B VJ and constant AA
MGIRLLCRVAFCFLAVGLVDVKVTQSSRYLVKRTGEKVFLECVQDMDHENMFWYRQDPGLGLRLIYFSYDVKMKEKGDIPEGYSVSREKKERFSLILESASTNQTSMYLCASTPWLAGGNEQFFGPGTRLTVLEDLKNVFPPEVAVFEPSEAEISHTQKATLVCLATGFYPDHVELSWVWNGKEVHSGVSTDPQPLKEQPALNDSRYCLSSRLRVSATFWQNPRNHFRCQVQFYGLSENDEWTQDRAKPVTQIVSAEAWGRADCGFTSESYQQGVLSATILYEILLGKATLYAVLVSALVLMAMVKRKDSRG

SEQ ID NO: 44 - protein, 306 aa, synthetic construct
  REGION 1..306: note = beta VJ and constant (murine) AA
MGIRLLCRVAFCFLAVGLVDVKVTQSSRYLVKRTGEKVFLECVQDMDHENMFWYRQDPGLGLRLIYFSYDVKMKEKGDIPEGYSVSREKKERFSLILESASTNQTSMYLCASTPWLAGGNEQFFGPGTRLTVLEDLRNVTPPKVSLFEPSKAEIANKQKATLVCLARGFFPDHVELSVWWNGKEVHSGVCTDPQAYKESNYSYCLSSRLRVSATFWHNPRNHFRCQVQFHGLSEEDKWPEGSPKPVTQNISAEAWGRADCGITSASYHQGVLSATILYEILLGKATLYAVLVSGLVLMAMVKKKNS

SEQ ID NO: 45 - DNA, 939 bp, synthetic construct
  source 1..939: mol_type = other DNA
  misc_feature 1..939: note = b VJ and constant NT
atgggaatcaggctcctctgtcgtgtggccttttgtttcctggctgtaggcctcgtagatgtgaaagtaacccagagctcgagatatctagtcaaaaggacgggagagaaagtttttctggaatgtgtccaggatatggaccatgaaaatatgttctggtatcgacaagacccaggtctggggctacggctgatctatttctcatatgatgttaaaatgaaagaaaaaggagatattcctgaggggtacagtgtctctagagagaagaaggagcgcttctccctgattctggagtccgccagcaccaaccagacatctatgtacctctgtgccagcaccccgtggctagcgggaggcaatgagcagttcttcgggccagggacacggctcaccgtgctagaggacctgaaaaacgtgttcccacccgaggtcgctgtgtttgagccatcagaagcagagatctcccacacccaaaaggccacactggtatgcctggccacaggcttctaccccgaccacgtggagctgagctggtgggtgaatgggaaggaggtgcacagtggggtcagcacagacccgcagcccctcaaggagcagcccgccctcaatgactccagatactgcctgagcagccgcctgagggtctcggccaccttctggcagaacccccgcaaccacttccgctgtcaagtccagttctacgggctctcggagaatgacgagtggacccaggatagggccaaacccgtcacccagatcgtcagcgccgaggcctggggtagagcagactgtggcttcacctccgagtcttaccagcaaggggtcctgtctgccaccatcctctatgagatcttgctagggaaggccaccttgtatgccgtgctggtcagtgccctcgtgctgatggccatggtcaagagaaaggattccagaggctag

SEQ ID NO: 46 - DNA, 939 bp, synthetic construct
  source 1..939: mol_type = other DNA
  misc_feature 1..939: note = b VJ and constant NT co
atgggcatccggctgctgtgcagagtggccttctgctttctggccgtgggcctggtggacgtgaaagtgacccagagcagcagatacctcgtgaagcggaccggcgagaaggtgttcctggaatgcgtgcaggacatggaccacgagaatatgttctggtacagacaggaccccggcctgggcctgcggctgatctacttcagctacgacgtgaagatgaaggaaaagggcgacatccccgagggctacagcgtgtccagagagaagaaagagcggttcagcctgatcctggaaagcgccagcaccaaccagaccagcatgtacctgtgtgccagcaccccttggctggctggcggcaacgagcagttttttggccctggcacccggctgaccgtgctggaagatctgaagaacgtgttccccccagaggtggccgtgttcgagccttctgaggccgagatcagccacacccagaaagccaccctcgtgtgtctggccaccggcttctaccccgaccacgtggaactgtcttggtgggtcaacggcaaagaggtgcacagcggcgtgtccaccgatccccagcctctgaaagaacagcccgccctgaacgacagccggtactgcctgtccagcagactgagagtgtccgccaccttctggcagaacccccggaaccacttcagatgccaggtgcagttctacggcctgagcgagaacgacgagtggacccaggacagagccaagcccgtgacacagatcgtgtctgccgaagcctggggcagagccgattgcggctttaccagcgagagctaccagcagggcgtgctgagcgccaccatcctgtacgagatcctgctgggcaaggccaccctgtacgccgtgctggtgtctgccctggtgctgatggccatggtcaagcggaaggacagccggggctaa

SEQ ID NO: 47 - skipped

SEQ ID NO: 48 - protein, 918 aa, synthetic construct
  REGION 1..918: note = b VJ and constant (murine) NT co
ATGGGCATCCGGCTGCTGTGCAGAGTGGCCTTCTGCTTTCTGGCCGTGGGCCTGGTGGACGTGAAAGTGACCCAGAGCAGCAGATACCTCGTGAAGCGGACCGGCGAGAAGGTGTTCCTGGAATGCGTGCAGGACATGGACCACGAGAATATGTTCTGGTACAGACAGGACCCCGGCCTGGGCCTGCGGCTGATCTACTTCAGCTACGACGTGAAGATGAAGGAAAAGGGCGACATCCCCGAGGGCTACAGCGTGTCCAGAGAGAAGAAAGAGCGGTTCAGCCTGATCCTGGAAAGCGCCAGCACCAACCAGACCAGCATGTACCTGTGTGCCAGCACCCCTTGGCTGGCTGGCGGCAACGAGCAGTTTTTTGGCCCTGGCACCCGGCTGACCGTGCTGGAAGATCTACGTAACGTGACACCACCCAAAGTCTCACTGTTTGAGCCTAGCAAGGCAGAAATTGCCAACAAGCAGAAGGCCACCCTGGTGTGCCTGGCAAGAGGGTTCTTTCCAGATCACGTGGAGCTGTCCTGGTGGGTCAACGGCAAAGAAGTGCATTCTGGGGTCTGCACCGACCCCCAGGCTTACAAGGAGAGTAATTACTCATATTGTCTGTCAAGCCGGCTGAGAGTGTCCGCCACATTCTGGCACAACCCTAGGAATCATTTCCGCTGCCAGGTCCAGTTTCACGGCCTGAGTGAGGAAGATAAATGGCCAGAGGGGTCACCTAAGCCAGTGACACAGAACATCAGCGCAGAAGCCTGGGGACGAGCAGACTGTGGCATTACTAGCGCCTCCTATCATCAGGGCGTGCTGAGCGCCACTATCCTGTACGAGATTCTGCTGGGAAAGGCCACCCTGTATGCTGTGCTGGTCTCCGGCCTGGTGCTGATGGCCATGGTCAAGAAAAAGAACTCT

SEQ ID NO: 49 - protein, 23 aa, synthetic construct
  REGION 1..23: note = a CDR3 AA
CAVKDNAGNMLTFGGGTRLMVKP

SEQ ID NO: 50 - DNA, 69 bp, synthetic construct
  source 1..69: mol_type = other DNA
  misc_feature 1..69: note = a CDR3 NT
tgtgccgtgaaggataatgcaggcaacatgctcacctttggagggggaacaaggttaatggtcaaaccc

SEQ ID NO: 51 - DNA, 69 bp, synthetic construct
  source 1..69: mol_type = other DNA
  misc_feature 1..69: note = a CDR3 NT co*
tgcgccgtgaaggacaacgccggcaacatgctgaccttcggcggaggcacccggctgatggtcaagccc

SEQ ID NO: 52 - protein, 23 aa, synthetic construct
  REGION 1..23: note = beta CDR3 AA
CASSDGGGVYEQYFGPGTRLTVT

SEQ ID NO: 53 - DNA, 69 bp, synthetic construct
  source 1..69: mol_type = other DNA
  misc_feature 1..69: note = b CDR3 NT
tgtgccagcagcgacggagggggcgtctacgagcagtacttcgggccgggcaccaggctcacggtcaca

SEQ ID NO: 54 - DNA, 69 bp, synthetic construct
  source 1..69: mol_type = other DNA
  misc_feature 1..69: note = b CDR3 NT co
tgtgccagctctgatggcggcggagtgtacgagcagtacttcggccctggcaccagactgaccgtgacc

SEQ ID NO: 55 - protein, 133 aa, synthetic construct
  REGION 1..133: note = a VJ AA
MMKSLRVLLVILWLQLSVWWSQQKEVEQNSGPLSVPEGAIASLNCTYSDRGSQSFFWYRQYSGKSPELIMFIYSNGDKEDGRFTAQLNKASQYVSLLIRDSQPSDSATYLCAVKDNAGNMLTFGGGTRLMVKP

SEQ ID NO: 56 - DNA, 399 bp, synthetic construct
  source 1..399: mol_type = other DNA
  misc_feature 1..399: note = a VJ NT
atgatgaaatccttgagagttttactagtgatcctgtggcttcagttgagctgggtttggagccaacagaaggaggtggagcagaattctggacccctcagtgttccagagggagccattgcctctctcaactgcacttacagtgaccgaggttcccagtccttcttctggtacagacaatattctgggaaaagccctgagttgataatgttcatatactccaatggtgacaaagaagatggaaggtttacagcacagctcaataaagccagccagtatgtttctctgctcatcagagactcccagcccagtgattcagccacctacctctgtgccgtgaaggataatgcaggcaacatgctcacctttggagggggaacaaggttaatggtcaaaccc

SEQ ID NO: 57 - DNA, 399 bp, synthetic construct
  source 1..399: mol_type = other DNA
  misc_feature 1..399: note = a VJ NT co
atgatgaagtccctgcgggtgctgctcgtgatcctgtggctgcagctgagctgggtgtggtcccagcagaaagaggtggaacagaacagcggccctctgagcgtgccagaaggcgctatcgccagcctgaactgcacctacagcgacagaggcagccagagcttcttctggtacagacagtacagcggcaagagccccgagctgatcatgttcatctacagcaacggcgacaaagaggacggccggttcaccgcccagctgaacaaggccagccagtacgtgtccctgctgatcagagacagccagcccagcgacagcgccacctatctgtgcgccgtgaaggacaacgccggcaacatgctgaccttcggcggaggcacccggctgatggtcaagccc

SEQ ID NO: 58 - protein, 132 aa, synthetic construct
  REGION 1..132: note = b VDJ AA
MGFRLLCCVAFCLLGAGPVDSGVTQTPKHLITATGQRVTLRCSPRSGDLSVYWYQQSLDQGLQFLIQYYNGEERAKGNILERFSAQQFPDLHSELNLSSLELGDSALYFCASSDGGGVYEQYFGPGTRLTVT

SEQ ID NO: 59 - DNA, 396 bp, synthetic construct
  source 1..396: mol_type = other DNA
  misc_feature 1..396: note = b VDJ NT
atgggcttcaggctcctctgctgtgtggccttttgtctcctgggagcaggcccagtggattctggagtcacacaaaccccaaagcacctgatcacagcaactggacagcgagtgacgctgagatgctcccctaggtctggagacctctctgtgtactggtaccaacagagcctggaccagggcctccagttcctcattcagtattataatggagaagagagagcaaaaggaaacattcttgaacgattctccgcacaacagttccctgacttgcactctgaactaaacctgagctctctggagctgggggactcagctttgtatttctgtgccagcagcgacggagggggcgtctacgagcagtacttcgggccgggcaccaggctcacggtcaca

SEQ ID NO: 60 - DNA, 396 bp, synthetic construct
  source 1..396: mol_type = other DNA
  misc_feature 1..396: note = b VDJ NT co
atgggcttcagactgctgtgctgcgtggccttctgtctgctgggagccggccctgtggatagcggcgtgacacagacacccaagcacctgatcaccgccaccggccagcgcgtgacactgagatgtagccctagaagcggcgacctgagcgtgtactggtatcagcagagcctggaccagggcctgcagttcctgatccagtactacaacggcgaggaacgggccaagggcaacatcctggaacggttcagcgcccagcagttccccgatctgcacagcgagctgaacctgagcagcctggaactgggcgacagcgccctgtacttctgtgccagctctgatggcggcggagtgtacgagcagtacttcggccctggcaccagactgaccgtgacc

SEQ ID NO: 61 - protein, 274 aa, synthetic construct
  REGION 1..274: note = a VJ and constant AA
MMKSLRVLLVILWLQLSVWWSQQKEVEQNSGPLSVPEGAIASLNCTYSDRGSQSFFWYRQYSGKSPELIMFIYSNGDKEDGRFTAQLNKASQYVSLLIRDSQPSDSATYLCAVKDNAGNMLTFGGGTRLMVKPHIQNPDPAVYQLRDSKSSDKSVCLFTDFDSQTNVSQSKDSDVYITDKTVLDMRSMDFKSNSAVAWSNKSDFACANAFNNSIIPEDTFFPSPESSCDVKLVEKSFETDTNLNFQNLSVIGFRILLLKVAGFNLLMTLRLWSS

SEQ ID NO: 62 - protein, 270 aa, synthetic construct
  REGION 1..270: note = a VJ and constant (murine) AA
MMKSLRVLLVILWLQLSVWWSQQKEVEQNSGPLSVPEGAIASLNCTYSDRGSQSFFWYRQYSGKSPELIMFIYSNGDKEDGRFTAQLNKASQYVSLLIRDSQPSDSATYLCAVKDNAGNMLTFGGGTRLMVKPDIQNPEPAVYQLKDPRSQDSTLCLFTDFDSQINVPKTMESGTFITDKCVLDMKAMDSKSNGAIAWSNQTSFTCQDIFKETNATYPSSDVPCDATLTEKSFETDMNLNFQNLSVMGLRILLLKVAGFNLLMTLRLWSS

SEQ ID NO: 63 - DNA, 825 bp, synthetic construct
  source 1..825: mol_type = other DNA
  misc_feature 1..825: note = a VJ and constant NT
atgatgaaatccttgagagttttactagtgatcctgtggcttcagttgagctgggtttggagccaacagaaggaggtggagcagaattctggacccctcagtgttccagagggagccattgcctctctcaactgcacttacagtgaccgaggttcccagtccttcttctggtacagacaatattctgggaaaagccctgagttgataatgttcatatactccaatggtgacaaagaagatggaaggtttacagcacagctcaataaagccagccagtatgtttctctgctcatcagagactcccagcccagtgattcagccacctacctctgtgccgtgaaggataatgcaggcaacatgctcacctttggagggggaacaaggttaatggtcaaaccccatatccagaaccctgaccctgccgtgtaccagctgagagactctaaatccagtgacaagtctgtctgcctattcaccgattttgattctcaaacaaatgtgtcacaaagtaaggattctgatgtgtatatcacagacaaaactgtgctagacatgaggtctatggacttcaagagcaacagtgctgtggcctggagcaacaaatctgactttgcatgtgcaaacgccttcaacaacagcattattccagaagacaccttcttccccagcccagaaagttcctgtgatgtcaagctggtcgagaaaagctttgaaacagatacgaacctaaactttcaaaacctgtcagtgattgggttccgaatcctcctcctgaaagtggccgggtttaatctgctcatgacgctgcggttgtggtccagctga

SEQ ID NO: 64 - DNA, 825 bp, synthetic construct
  source 1..825: mol_type = other DNA
  misc_feature 1..825: note = a VJ and constant NT co
atgatgaagtccctgcgggtgctgctcgtgatcctgtggctgcagctgagctgggtgtggtcccagcagaaagaggtggaacagaacagcggccctctgagcgtgccagaaggcgctatcgccagcctgaactgcacctacagcgacagaggcagccagagcttcttctggtacagacagtacagcggcaagagccccgagctgatcatgttcatctacagcaacggcgacaaagaggacggccggttcaccgcccagctgaacaaggccagccagtacgtgtccctgctgatcagagacagccagcccagcgacagcgccacctatctgtgcgccgtgaaggacaacgccggcaacatgctgaccttcggcggaggcacccggctgatggtcaagccccacatccagaaccccgaccccgccgtgtaccagctgagagacagcaagagcagcgataagagcgtgtgcctgttcaccgacttcgacagccagaccaacgtgtcccagagcaaggacagcgacgtgtacatcaccgacaagaccgtgctggacatgcggagcatggacttcaagagcaacagcgccgtggcctggtccaacaagagcgatttcgcctgcgccaacgccttcaacaacagcattatccccgaggacacattcttcccaagccccgagagcagctgcgacgtgaagctggtggaaaagagcttcgagacagacaccaacctgaacttccagaacctgagcgtgatcggcttccggatcctgctgctgaaggtggccggcttcaacctgctgatgaccctgagactgtggtccagctga

SEQ ID NO: 65 - skipped

SEQ ID NO: 66 - DNA, 813 bp, synthetic construct
  source 1..813: mol_type = other DNA
  misc_feature 1..813: note = a VJ and constant (murine) NT co
atgatgaagtccctgcgggtgctgctcgtgatcctgtggctgcagctgagctgggtgtggtcccagcagaaagaggtggaacagaacagcggccctctgagcgtgccagaaggcgctatcgccagcctgaactgcacctacagcgacagaggcagccagagcttcttctggtacagacagtacagcggcaagagccccgagctgatcatgttcatctacagcaacggcgacaaagaggacggccggttcaccgcccagctgaacaaggccagccagtacgtgtccctgctgatcagagacagccagcccagcgacagcgccacctatctgtgcgccgtgaaggacaacgccggcaacatgctgaccttcggcggaggcacccggctgatggtcaagcccgacattcagaacccggaaccggctgtataccagctgaaggacccccgatctcaggatagtactctgtgcctgttcaccgactttgatagtcagatcaatgtgcctaaaaccatggaatccggaacttttattaccgacaagtgcgtgctggatatgaaagccatggacagtaagtcaaacggcgccatcgcttggagcaatcagacatccttcacttgccaggatatcttcaaggagaccaacgcaacatacccatcctctgacgtgccctgtgatgccaccctgacagagaagtctttcgaaacagacatgaacctgaattttcagaatctgagcgtgatgggcctgagaatcctgctgctgaaggtcgctgggtttaatctgctgatgacactgcggctgtggtcctcatga

SEQ ID NO: 67 - protein, 311 aa, synthetic construct
  REGION 1..311: note = b VJ and constant AA
MGFRLLCCVAFCLLGAGPVDSGVTQTPKHLITATGQRVTLRCSPRSGDLSVYWYQQSLDQGLQFLIQYYNGEERAKGNILERFSAQQFPDLHSELNLSSLELGDSALYFCASSDGGGVYEQYFGPGTRLTVTEDLKNVFPPEVAVFEPSEAEISHTQKATLVCLATGFYPDHVELSVWWNGKEVHSGVSTDPQPLKEQPALNDSRYCLSSRLRVSATFWQNPRNHFRCQVQFYGLSENDEWTQDRAKPVTQIVSAEAWGRADCGFTSESYQQGVLSATILYEILLGKATLYAVLVSALVLMAMVKRKDSRG

SEQ ID NO: 68 - protein, 305 aa, synthetic construct
  REGION 1..305: note = b VJ and constant (murine) AA
MGFRLLCCVAFCLLGAGPVDSGVTQTPKHLITATGQRVTLRCSPRSGDLSVYWYQQSLDQGLQFLIQYYNGEERAKGNILERFSAQQFPDLHSELNLSSLELGDSALYFCASSDGGGVYEQYFGPGTRLTVTEDLRNVTPPKVSLFEPSKAEIANKQKATLVCLARGFFPDHVELSVWWNGKEVHSGVCTDPQAYKESNYSYCLSSRLRVSATFWHNPRNHFRCQVQFHGLSEEDKWPEGSPKPVTQNISAEAWGRADCGITSASYHQGVLSATILYEILLGKATLYAVLVSGLVLMAMVKKKNS

SEQ ID NO: 69 - DNA, 936 bp, synthetic construct
  source 1..936: mol_type = other DNA
  misc_feature 1..936: note = b VJ and constant NT
atgggcttcaggctcctctgctgtgtggccttttgtctcctgggagcaggcccagtggattctggagtcacacaaaccccaaagcacctgatcacagcaactggacagcgagtgacgctgagatgctcccctaggtctggagacctctctgtgtactggtaccaacagagcctggaccagggcctccagttcctcattcagtattataatggagaagagagagcaaaaggaaacattcttgaacgattctccgcacaacagttccctgacttgcactctgaactaaacctgagctctctggagctgggggactcagctttgtatttctgtgccagcagcgacggagggggcgtctacgagcagtacttcgggccgggcaccaggctcacggtcacagaggacctgaaaaacgtgttcccacccgaggtcgctgtgtttgagccatcagaagcagagatctcccacacccaaaaggccacactggtatgcctggccacaggcttctaccccgaccacgtggagctgagctggtgggtgaatgggaaggaggtgcacagtggggtcagcacagacccgcagcccctcaaggagcagcccgccctcaatgactccagatactgcctgagcagccgcctgagggtctcggccaccttctggcagaacccccgcaaccacttccgctgtcaagtccagttctacgggctctcggagaatgacgagtggacccaggatagggccaaacccgtcacccagatcgtcagcgccgaggcctggggtagagcagactgtggcttcacctccgagtcttaccagcaaggggtcctgtctgccaccatcctctatgagatcttgctagggaaggccaccttgtatgccgtgctggtcagtgccctcgtgctgatggccatggtcaagagaaaggattccagaggctag

SEQ ID NO: 70 - DNA, 936 bp, synthetic construct
  source 1..936: mol_type = other DNA
  misc_feature 1..936: note = b VJ and constant NT co
atgggcttcagactgctgtgctgcgtggccttctgtctgctgggagccggccctgtggatagcggcgtgacacagacacccaagcacctgatcaccgccaccggccagcgcgtgacactgagatgtagccctagaagcggcgacctgagcgtgtactggtatcagcagagcctggaccagggcctgcagttcctgatccagtactacaacggcgaggaacgggccaagggcaacatcctggaacggttcagcgcccagcagttccccgatctgcacagcgagctgaacctgagcagcctggaactgggcgacagcgccctgtacttctgtgccagctctgatggcggcggagtgtacgagcagtacttcggccctggcaccagactgaccgtgaccgaggacctgaagaacgtgttccccccagaggtggccgtgttcgagccttctgaggccgagatcagccacacccagaaagccaccctcgtgtgtctggccaccggcttctaccccgaccacgtggaactgtcttggtgggtcaacggcaaagaggtgcacagcggcgtgtccaccgatccccagcctctgaaagaacagcccgccctgaacgacagccggtactgcctgtccagcagactgagagtgtccgccaccttctggcagaacccccggaaccacttcagatgccaggtgcagttctacggcctgagcgagaacgacgagtggacccaggacagagccaagcccgtgacccagatcgtgtctgccgaagcctggggcagagccgattgcggctttaccagcgagagctaccagcagggcgtgctgagcgccaccatcctgtacgagatcctgctgggcaaggccaccctgtacgccgtgctggtgtctgccctggtgctgatggccatggtcaagcggaaggacagccggggctaa

SEQ ID NO: 71 - skipped

SEQ ID NO: 72 - DNA, 915 bp, synthetic construct
  source 1..915: mol_type = other DNA
  misc_feature 1..915: note = b VJ and constant (murine) NT co
atgggcttcagactgctgtgctgcgtggccttctgtctgctgggagccggccctgtggatagcggcgtgacacagacacccaagcacctgatcaccgccaccggccagcgcgtgacactgagatgtagccctagaagcggcgacctgagcgtgtactggtatcagcagagcctggaccagggcctgcagttcctgatccagtactacaacggcgaggaacgggccaagggcaacatcctggaacggttcagcgcccagcagttccccgatctgcacagcgagctgaacctgagcagcctggaactgggcgacagcgccctgtacttctgtgccagctctgatggcggcggagtgtacgagcagtacttcggccctggcaccagactgaccgtgaccgaagatctacgtaacgtgacaccacccaaagtctcactgtttgagcctagcaaggcagaaattgccaacaagcagaaggccaccctggtgtgcctggcaagagggttctttccagatcacgtggagctgtcctggtgggtcaacggcaaagaagtgcattctggggtctgcaccgacccccaggcttacaaggagagtaattactcatattgtctgtcaagccggctgagagtgtccgccacattctggcacaaccctaggaatcatttccgctgccaggtccagtttcacggcctgagtgaggaagataaatggccagaggggtcacctaagccagtgacacagaacatcagcgcagaagcctggggacgagcagactgtggcattactagcgcctcctatcatcagggcgtgctgagcgccactatcctgtacgagattctgctgggaaaggccaccctgtatgctgtgctggtctccggcctggtgctgatggccatggtcaagaaaaagaactct

SEQ ID NO: 73 - skipped

SEQ ID NO: 74 - DNA, 846 bp, Homo sapiens
  source 1..846: mol_type = unassigned DNA
ggatttggtgatgtcggtgctcttgagagtttgaggggaaatgcagatttggcttacatcctgagcatggagccctgtggccactgcctcattatcaacaatgtgaacttctgccgtgagtccgggctccgcacccgcactggctccaacatcgactgtgagaagttgcggcgtcgcttctcctcgctgcatttcatggtggaggtgaagggcgacctgactgccaagaaaatggtgctggctttgctggagctggcgcagcaggaccacggtgctctggactgctgcgtggtggtcattctctctcacggctgtcaggccagccacctgcagttcccaggggctgtctacggcacagatggatgccctgtgtcggtcgagaagattgtgaacatcttcaatgggaccagctgccccagcctgggagggaagcccaagctctttttcatccaggcctgtggtggggagcagaaagaccatgggtttgaggtggcctccacttcccctgaagacgagtcccctggcagtaaccccgagccagatgccaccccgttccaggaaggtttgaggaccttcgaccagctggacgccatatctagtttgcccacacccagtgacatctttgtgtcctactctactttcccaggttttgtttcctggagggaccccaagagtggctcctggtacgttgagaccctggacgacatctttgagcagtgggctcactctgaagacctgcagtccctcctgcttagggtcgctaatgctgtttcggtgaaagggatttataaacagatgcctggttgctttaatttcctccggaaaaaacttttctttaaaacatca

SEQ ID NO: 75 - protein, 282 aa, Homo sapiens
GFGDVGALESLRGNADLAYILSMEPCGHCLIINNVNFCRESGLRTRTGSNIDCEKLRRRFSSLHFMVEVKGDLTAKKMVLALLELAQQDHGALDCCVVVILSHGCQASHLQFPGAVYGTDGCPVSVEKIVNIFNGTSCPSLGGKPKLFFIQACGGEQKDHGFEVASTSPEDESPGSNPEPDATPFQEGLRTFDQLDAISSLPTPSDIFVSYSTFPGFVSWRDPKSGSWYVETLDDIFEQWAHSEDLQSLLLRVANAVSVKGIYKQMPGCFNFLRKKLFFKTS

SEQ ID NO: 76 - DNA, 321 bp, synthetic construct
  source 1..321: mol_type = other DNA
  misc_feature 1..321: note = FKBPv36 (Fv1) nucleotide sequence
ggcgttcaagtagaaacaatcagcccaggagacggaaggactttccccaaacgaggccaaacatgcgtagttcattatactgggatgctcgaagatggaaaaaaagtagatagtagtagagaccgaaacaaaccatttaaatttatgttgggaaaacaagaagtaataaggggctgggaagaaggtgtagcacaaatgtctgttggccagcgcgcaaaactcacaatttctcctgattatgcttacggagctaccggccaccccggcatcataccccctcatgccacactggtgtttgacgtcgaattgctcaaactggaa

SEQ ID NO: 77 - protein, 106 aa, synthetic construct
  REGION 1..106: note = FKBPv36 (Fv1) amino acid sequence
GVQVETISPGDGRTFPKRGQTCWHYTGMLEDGKKVDSSRDRNKPFKFMLGKQEVIRGWEEGVAQMSVGQRAKLTISPDYAYGATGHPGIIPPHATLVFDVELLKLE

SEQ ID NO: 78 - DNA, 321 bp, synthetic construct
  source 1..321: mol_type = other DNA
  misc_feature 1..321: note = FKBPv36 (Fv2) nucleotide sequence
ggagtgcaggtggagacgattagtcctggggatgggagaacctttccaaagcgcggtcagacctgtgttgtccactacaccggtatgctggaggacgggaagaaggtggactcttcacgcgatcgcaataagcctttcaagttcatgctcggcaagcaggaggtgatccgggggtgggaggagggcgtggctcagatgtcggtcgggcaacgagcgaagcttaccatctcacccgactacgcgtatggggcaacggggcatccgggaattatccctccccacgctacgctcgtattcgatgtggagctcttgaagcttgag

SEQ ID NO: 79 - protein, 106 aa, synthetic construct; identical to SEQ ID NO: 77
  REGION 1..106: note = FKBPv36 (Fv2) amino acid sequence

SEQ ID NO: 80 - DNA, 54 bp, synthetic construct
  source 1..54: mol_type = other DNA
  misc_feature 1..54: note = T2A.codon optimized nucleotide sequence
gaaggccgagggagcctgctgacatgtggcgatgtggaggaaaacccaggacca

SEQ ID NO: 81 - protein, 18 aa, synthetic construct
  REGION 1..18: note = T2A.codon optimized amino acid sequence
EGRGSLLTCGDVEENPGP

SEQ ID NO: 82 - DNA, 57 bp, Thosea asigna virus
  source 1..57: mol_type = unassigned DNA
gccgagggcaggggaagtcttctaacatgcggggacgtggaggaaaatcccgggccc

SEQ ID NO: 83 - protein, 19 aa, Thosea asigna virus
AEGRGSLLTCGDVEENPGP

SEQ ID NO: 84 - protein, 106 aa, synthetic construct
  REGION 1..106: note = FKBP amino acid sequence (with phenylalanine at position 36)
GVQVETISPGDGRTFPKRGQTCWHYTGMLEDGKKFDSSRDRNKPFKFMLGKQEVIRGWEEGVAQMSVGQRAKLTISPDYAYGATGHPGIIPPHATLVFDVELLKLE

SEQ ID NO: 85 - DNA, 9433 bp, synthetic construct
  source 1..9433: mol_type = other DNA
  misc_feature 1..9433: note = SFG.iC9-2A-SLL.TCR iCasp9-PRAME TCR Coding Sequence
tgaaagaccccacctgtaggtttggcaagctagcttaagtaacgccattttgcaaggcatggaaaaatacataactgagaatagaaaagttcagatcaaggtcaggaacagatggaacagctgaatatgggccaaacaggatatctgtggtaagcagttcctgccccggctcagggccaagaacagatggaacagctgaatatgggccaaacaggatatctgtggtaagcagttcctgccccggctcagggccaagaacagatggtccccagatgcggtccagccctcagcagtttctagagaaccatcagatgtttccagggtgccccaaggacctgaaatgaccctgtgccttatttgaactaaccaatcagttcgcttctcgcttctgttcgcgcgcttatgctccccgagctcaataaaagagcccacaacccctcactcggggcgccagtcctccgattgactgagtcgcccgggtacccgtgtatccaataaaccctcttgcagttgcatccgacttgtggtctcgctgttccttgggagggtctcctctgagtgattgactacccgtcagcgggggtctttcatttgggggctcgtccgggatcgggagacccctgcccagggaccaccgacccaccaccgggaggtaagctggccagcaacttatctgtgtctgtccgattgtctagtgtctatgactgattttatgcgcctgcgtcggtactagttagctaactagctctgtatctggcggacccgtggtggaactgacgagttcggaacacccggccgcaaccctgggagacgtcccagggacttcgggggccgtttttgtggcccgacctgagtcctaaaatcccgatcgtttaggactctttggtgcaccccccttagaggagggatatgtggttctggtaggagacgagaacctaaaacagttcccgcctccgtctgaatttttgctttcggtttgggaccgaagccgcgccgcgcgtcttgtctgctgcagcatcgttctgtgttgtctctgtctgactgtgtttctgtatttgtctgaaaatatgggcccgggctagcctgttaccactcccttaagtttgaccttaggtcactggaaagatgtcgagcggatcgctcacaaccagtcggtagatgtcaagaagagacgttgggttaccttctgctctgcagaatggccaacctttaacgtcggatggccgcgagacggcacctttaaccgagacctcatcacccaggttaagatcaaggtcttttcacctggcccgcatggacacccagaccaggtggggtacatcgtgacctgggaagccttggcttttgacccccctccctgggtcaagccctttgtacaccctaagcctccgcctcctcttcctccatccgccccgtctctcccccttgaacctcctcgttcgaccccgcctcgatcctccctttatccagccctcactccttctctaggcgcccccatatggccatatgagatcttatatggggcacccccgccccttgtaaacttccctgaccctgacatgacaagagttactaacagcccctctctccaagctcacttacaggctctctacttagtccagcacgaagtctggagacctctggcggcagcctaccaagaacaactggaccgaccggtggtacctcacccttaccgagtcggcgacacagtgtgggtccgccgacaccagactaagaacctagaacctcgctggaaaggaccttacacagtcctgctgaccacccccaccgccctcaaagtagacggcatcgcagcttggatacacgccgcccacgtgaaggctgccgaccccgggggtggaccatcctctagactgccatgctcgagggagtgcaggtggaaaccatctccccaggagacgggcgcaccttccccaagcgcggccagacctgcgtggtgcactacaccgggatgcttgaagatggaaagaaagttgattcctcccgggacagaaacaagccctttaagtttatgctaggcaagcaggaggtgatccgaggctgggaagaaggggttgcccagatgagtgtgggtcagagagccaaactgactatatctccagattatgcctatggtgccactgggcacccaggcatcatcccaccacatgccactctcgtcttcgatgtggagcttctaaaactggaatctggcggtggatccggagtcgacggatttggtgatgtcggtgctcttgagagtttgaggggaaatgcagatttggcttacatcctgagcatggagccctgtggccactgcctcattatcaacaatgtgaacttctgccgtgagtccgggctccgcacccgcactggctccaacatcgactgtgagaagttgcggcgtcgcttctcctcgctgcatttcatggtggaggtgaagggcgacctgactgccaagaaaatggtgctggctttgctggagctggcgcagcaggaccacggtgctctggactgctgcgtggtggtcattctctctcacggctgtcaggccagccacctgcagttcccaggggctgtctacggcacagatggatgccctgtgtcggtcgagaagattgtgaacatcttcaatgggaccagctgccccagcctgggagggaagcccaagctctttttcatccaggcctgtggtggggagcagaaagaccatgggtttgaggtggcctccacttcccctgaagacgagtcccctggcagtaaccccgagccagatgccaccccgttccaggaaggtttgaggaccttcgaccagctggacgccatatctagtttgcccacacccagtgacatctttgtgtcctactctactttcccaggttttgtttcctggagggaccccaagagtggctcctggtacgttgagaccctggacgacatctttgagcagtgggctcactctgaagacctgcagtccctcctgcttagggtcgctaatgctgtttcggtgaaagggatttataaacagatgcctggttgctttaatttcctccggaaaaaacttttctttaaaacatcagctagcagagccgagggcaggggaagtcttctaacatgcggggacgtggaggaaaatcccgggcccatgggcttccggctgctgtgctgcgtggccttttgtctgctgggagccggccctgtggatagcggcgtgacccagacccccaagcacctgatcaccgccaccggccagagagtgaccctgcgctgcagccctagaagcggcgacctgagcgtgtactggtatcagcagagcctcgaccagggcctgcagttcctgatccagtactacaacggcgaggaacgggccaagggcaacatcctggaacggttcagcgcccagcagttccccgatctgcacagcgagctgaacctgagcagcctggaactgggcgacagcgccctgtacttctgcgccagcgccagatgggatagaggcggcgagcagtacttcggccctggcaccagactgaccgtgaccgaggacctgaagaacgtgttccccccagaggtggccgtgtttgagcccagcgaggccgagatcagccacacccagaaagccaccctggtgtgcctggccaccggcttctaccccgaccacgtggagctgtcttggtgggtgaacggcaaagaggtgcacagcggcgtctgcaccgacccccagcccctgaaagagcagcccgccctgaacgacagccggtactgcctgagcagcagactgcgggtgtccgccaccttctggcagaacccccggaaccacttccggtgccaggtgcagttctacggcctgagcgagaacgacgagtggacccaggacagagccaagcctgtgacccagatcgtgtctgccgaagcctggggcagagccgactgcggcttcaccagcgagagctaccagcagggcgtgctgagcgccaccatcctgtacgagatcctgctgggcaaggccacactgtacgccgtgctggtgtccgctctggtgctgatggccatggtgaagcggaaggacagcagaggcgagggcagaggaagtcttctaacatgcggtgacgtggaggagaatcccggccctatgctgctgctgctggtgcccgtgctggaagtgatcttcaccctgggcggcaccagagcccagagcgtgacacagctgggcagccacgtgtccgtgtctgagagggccctggtgctgctgagatgcaactactcttctagcgtgcccccctacctgttttggtacgtgcagtaccccaaccaggggctgcagctgctcctgaagtacaccagcgccgccacactggtgaagggcatcaacggcttcgaggccgagttcaagaagtccgagacaagcttccacctgaccaagcccagcgcccacatgtctgacgccgccgagtacttctgtgccgtgagcggccagaccggcgccaacaacctgttcttcggcaccggcacccggctgacagtgatcccttacatccagaaccccgaccccgccgtgtaccagctgcgggacagcaagagcagcgacaagagcgtgtgcctgttcaccgacttcgacagccagaccaacgtgtcccagagcaaggacagcgacgtgtacatcaccgataagtgcgtgctggacatgcggagcatggacttcaagagcaacagcgccgtggcctggtccaacaagagcgacttcgcctgcgccaacgccttcaacaacagcatcatccccgaggacacattcttcccaagccccgagagcagctgcgacgtgaagctggtggagaagtccttcgagacagacaccaacctgaacttccagaacctgtccgtgatcggcttcagaatcctgctgctgaaagtggccggcttcaacctgctgatgaccctgcggctgtggtccagctgaacgcgtcatcatcgatccggattagtccaatttgttaaagacaggatatcagtggtccaggctctagttttgactcaacaatatcaccagctgaagcctatagagtacgagccatagataaaataaaagattttatttagtctccagaaaaaggggggaatgaaagaccccacctgtaggtttggcaagctagcttaagtaacgccattttgcaaggcatggaaaaatacataactgagaatagagaagttcagatcaaggtcaggaacagatggaacagctgaatatgggccaaacaggatatctgtggtaagcagttcctgccccggctcagggccaagaacagatggaacagctgaatatgggccaaacaggatatctgtggtaagcagttcctgccccggctcagggccaagaacagatggtccccagatgcggtccagccctcagcagtttctagagaaccatcagatgtttccagggtgccccaaggacctgaaatgaccctgtgccttatttgaactaaccaatcagttcgcttctcgcttctgttcgcgcgcttctgctccccgagctcaataaaagagcccacaacccctcactcggggcgccagtcctccgattgactgagtcgcccgggtacccgtgtatccaataaaccctcttgcagttgcatccgacttgtggtctcgctgttccttgggagggtctcctctgagtgattgactacccgtcagcgggggtctttcacacatgcagcatgtatcaaaattaatttggttttttttcttaagtatttacattaaatggccatagtacttaaagttacattggcttccttgaaataaacatggagtattcagaatgtgtcataaatatttctaattttaagatagtatctccattggctttctactttttcttttatttttttttgtcctctgtcttccatttgttgttgttgttgtttgtttgtttgtttgttggttggttggttaatttttttttaaagatcctacactatagttcaagctagactattagctactctgtaacccagggtgaccttgaagtcatgggtagcctgctgttttagccttcccacatctaagattacaggtatgagctatcatttttggtatattgattgattgattgattgatgtgtgtgtgtgtgattgtgtttgtgtgtgtgactgtgaaaatgtgtgtatgggtgtgtgtgaatgtgtgtatgtatgtgtgtgtgtgagtgtgtgtgtgtgtgtgtgcatgtgtgtgtgtgtgactgtgtctatgtgtatgactgtgtgtgtgtgtgtgtgtgtgtgtgtgtgtgtgtgtgtgtgtgtgttgtgaaaaaatattctatggtagtgagagccaacgctccggctcaggtgtcaggttggtttttgagacagagtctttcacttagcttggaattcactggccgtcgttttacaacgtcgtgactgggaaaaccctggcgttacccaacttaatcgccttgcagcacatccccctttcgccagctggcgtaatagcgaagaggcccgcaccgatcgcccttcccaacagttgcgcagcctgaatggcgaatggcgcctgatgcggtattttctccttacgcatctgtgcggtatttcacaccgcatatggtgcactctcagtacaatctgctctgatgccgcatagttaagccagccccgacacccgccaacacccgctgacgcgccctgacgggcttgtctgctcccggcatccgcttacagacaagctgtgaccgtctccgggagctgcatgtgtcagaggttttcaccgtcatcaccgaaacgcgcgatgacgaaagggcctcgtgatacgcctatttttataggttaatgtcatgataataatggtttcttagacgtcaggtggcacttttcggggaaatgtgcgcggaacccctatttgtttatttttctaaatacattcaaatatgtatccgctcatgagacaataaccctgataaatgcttcaataatattgaaaaaggaagagtatgagtattcaacatttccgtgtcgcccttattcccttttttgcggcattttgccttcctgtttttgctcacccagaaacgctggtgaaagtaaaagatgctgaagatcagttgggtgcacgagtgggttacatcgaactggatctcaacagcggtaagatccttgagagttttcgccccgaagaacgttttccaatgatgagcacttttaaagttctgctatgtggcgcggtattatcccgtattgacgccgggcaagagcaactcggtcgccgcatacactattctcagaatgacttggttgagtactcaccagtcacagaaaagcatcttacggatggcatgacagtaagagaattatgcagtgctgccataaccatgagtgataacactgcggccaacttacttctgacaacgatcggaggaccgaaggagctaaccgcttttttgcacaacatgggggatcatgtaactcgccttgatcgttgggaaccggagctgaatgaagccataccaaacgacgagcgtgacaccacgatgcctgtagcaatggcaacaacgttgcgcaaactattaactggcgaactacttactctagcttcccggcaacaattaatagactggatggaggcggataaagttgcaggaccacttctgcgctcggcccttccggctggctggtttattgctgataaatctggagccggtgagcgtgggtctcgcggtatcattgcagcactggggccagatggtaagccctcccgtatcgtagttatctacacgacggggagtcaggcaactatggatgaacgaaatagacagatcgctgagataggtgcctcactgattaagcattggtaactgtcagaccaagtttactcatatatactttagattgatttaaaacttcatttttaatttaaaaggatctaggtgaagatcctttttgataatctcatgaccaaaatcccttaacgtgagttttcgttccactgagcgtcagaccccgtagaaaagatcaaaggatcttcttgagatcctttttttctgcgcgtaatctgctgcttgcaaacaaaaaaaccaccgctaccagcggtggtttgtttgccggatcaagagctaccaactctttttccgaaggtaactggcttcagcagagcgcagataccaaatactgtccttctagtgtagccgtagttaggccaccacttcaagaactctgtagcaccgcctacatacctcgctctgctaatcctgttaccagtggctgctgccagtggcgataagtcgtgtcttaccgggttggactcaagacgatagttaccggataaggcgcagcggtcgggctgaacggggggttcgtgcacacagcccagcttggagcgaacgacctacaccgaactgagatacctacagcgtgagcattgagaaagcgccacgcttcccgaagggagaaaggcggacaggtatccggtaagcggcagggtcggaacaggagagcgcacgagggagcttccagggggaaacgcctggtatctttatagtcctgtcgggtttcgccacctctgacttgagcgtcgatttttgtgatgctcgtcaggggggcggagcctatggaaaaacgccagcaacgcggcctttttacggttcctggccttttgctggccttttgctcacatgttctttcctgcgttatcccctgattctgtggataaccgtattaccgcctttgagtgagctgataccgctcgccgcagccgaacgaccgagcgcagcgagtcagtgagcgaggaagcggaagagcgcccaatacgcaaaccgcctctccccgcgcgttggccgattcattaatgcagctggcacgacaggtttcccgactggaaagcgggcagtgagcgcaacgcaattaatgtgagttagctcactcattaggcaccccaggctttacactttatgcttccggctcgtatgttgtgtggaattgtgagcggataacaatttcacacaggaaacagctatgaccatgattacgccaagctttgctcttaggagtttcctaatacatcccaaactcaaatatataaagcatttgacttgttctatgccctagggggcggggggaagctaagccagctttttttaacatttaaaatgttaattccattttaaatgcacagatgtttttatttcataagggtttcaatgtgcatgaatgctgcaatattcctgttaccaaagctagtataaataaaaatagataaacgtggaaattacttagagtttctgtcattaacgtttccttcctcagttgacaacataaatgcgctgctgagcaagccagtttgcatctgtcaggatcaatttcccattatgccagtcatattaattactagtcaattagttgatttttatttttgacatatacatgtgaa

SEQ ID NO: 86 - DNA, 864 bp, synthetic construct
  source 1..864: mol_type = other DNA
  misc_feature 1..864: note = Nucleotide sequence coding for Caspase-9 polypeptide in SEQ ID NO: 85
gtcgacggatttggtgatgtcggtgctcttgagagtttgaggggaaatgcagatttggcttacatcctgagcatggagccctgtggccactgcctcattatcaacaatgtgaacttctgccgtgagtccgggctccgcacccgcactggctccaacatcgactgtgagaagttgcggcgtcgcttctcctcgctgcatttcatggtggaggtgaagggcgacctgactgccaagaaaatggtgctggctttgctggagctggcgcagcaggaccacggtgctctggactgctgcgtggtggtcattctctctcacggctgtcaggccagccacctgcagttcccaggggctgtctacggcacagatggatgccctgtgtcggtcgagaagattgtgaacatcttcaatgggaccagctgccccagcctgggagggaagcccaagctctttttcatccaggcctgtggtggggagcagaaagaccatgggtttgaggtggcctccacttcccctgaagacgagtcccctggcagtaaccccgagccagatgccaccccgttccaggaaggtttgaggaccttcgaccagctggacgccatatctagtttgcccacacccagtgacatctttgtgtcctactctactttcccaggttttgtttcctggagggaccccaagagtggctcctggtacgttgagaccctggacgacatctttgagcagtgggctcactctgaagacctgcagtccctcctgcttagggtcgctaatgctgtttcggtgaaagggatttataaacagatgcctggttgctttaatttcctccggaaaaaacttttctttaaaacatcagctagcagagcc

SEQ ID NO: 87 - DNA, 933 bp, synthetic construct; identical to SEQ ID NO: 22
  source 1..933: mol_type = other DNA
  misc_feature 1..933: note = Nucleotide sequence coding for TCR beta in SEQ ID NO: 85

SEQ ID NO: 88 - DNA, 822 bp, synthetic construct
  source 1..822: mol_type = other DNA
  misc_feature 1..822: note = Nucleotide sequence coding for TCR alpha in SEQ ID NO: 85
atgctgctgctgctggtgcccgtgctggaagtgatcttcaccctgggcggcaccagagcccagagcgtgacacagctgggcagccacgtgtccgtgtctgagagggccctggtgctgctgagatgcaactactcttctagcgtgcccccctacctgttttggtacgtgcagtaccccaaccaggggctgcagctgctcctgaagtacaccagcgccgccacactggtgaagggcatcaacggcttcgaggccgagttcaagaagtccgagacaagcttccacctgaccaagcccagcgcccacatgtctgacgccgccgagtacttctgtgccgtgagcggccagaccggcgccaacaacctgttcttcggcaccggcacccggctgacagtgatcccttacatccagaaccccgaccccgccgtgtaccagctgcgggacagcaagagcagcgacaagagcgtgtgcctgttcaccgacttcgacagccagaccaacgtgtcccagagcaaggacagcgacgtgtacatcaccgataagtgcgtgctggacatgcggagcatggacttcaagagcaacagcgccgtggcctggtccaacaagagcgacttcgcctgcgccaacgccttcaacaacagcatcatccccgaggacacattcttcccaagccccgagagcagctgcgacgtgaagctggtggagaagtccttcgagacagacaccaacctgaacttccagaacctgtccgtgatcggcttcagaatcctgctgctgaaagtggccggcttcaacctgctgatgaccctgcggctgtggtccagc

SEQ ID NO: 89 - protein, 274 aa, synthetic construct
  REGION 1..274: note = PRAME clone 54SLL
MLLLLVPVLEVIFTLGGTRAQSVTQLGSHVSVSERALVLLRCNYSSSVPPYLFWYVQYPNQGLQLLLKYTSAATLVKGINGFEAEFKKSETSFHLTKPSAHMSDAAEYFCAVSGQTGANNLFFGTGTRLTVIPYIQNPDPAVYQLRDSKSSDKSVCLFTDFDSQTNVSQSKDSDVYITDKTVLDMRSMDFKSNSAVAWSNKSDFACANAFNNSIIPEDTFFPSPESSCDVKLVEKSFETDTNLNFQNLSVIGFRILLLKVAGFNLLMTLRLWSS

SEQ ID NO: 90 - protein, 311 aa, synthetic construct
  REGION 1..311: note = PRAME clone 54SLL
MGFRLLCCVAFCLLGAGPVDSGVTQTPKHLITATGQRVTLRCSPRSGDLSVYWYQQSLDQGLQFLIQYYNGEERAKGNILERFSAQQFPDLHSELNLSSLELGDSALYFCASARWDRGGEQYFGPGTRLTVTEDLKNVFPPEVAVFEPSEAEISHTQKATLVCLATGFYPDHVELSWWVNGKEVHSGVSTDPQPLKEQPALNDSRYCLSSRLRVSATFWQNPRNHFRCQVQFYGLSENDEWTQDRAKPVTQIVSAEAWGRADCGFTSESYQQGVLSATILYEILLGKATLYAVLVSALVLMAMVKRKDSRG

SEQ ID NO: 91 - protein, 272 aa, synthetic construct
  REGION 1..272: note = PRAME clone 46SLL
MLLEHLLIILWMQLTWVSGQQLNQSPQSMFIQEGEDVSMNCTSSSIFNTWLWYKQDPGEGPVLLIALYKAGELTSNGRLTAQFGITRKDSFLNISASIPSDVGIYFCAGIPRDNYGQNFVFGPGTRLSVLPYIQNPDPAVYQLRDSKSSDKSVCLFTDFDSQTNVSQSKDSDVYITDKTVLDMRSMDFKSNSAVAWSNKSDFACANAFNNSIIPEDTFFPSPESSCDVKLVEKSFETDTNLNFQNLSVIGFRILLLKVAGFNLLMTLRLWSS

SEQ ID NO: 92 - protein, 312 aa, synthetic construct
  REGION 1..312: note = PRAME clone 46SLL
MGIRLLCRVAFCFLAVGLVDVKVTQSSRYLVKRTGEKVFLECVQDMDHENMFWYRQDPGLGLRLIYFSYDVKMKEKGDIPEGYSVSREKKERFSLILESASTNQTSMYLCASTPWLAGGNEQFFGPGTRLTVLEDLKNVFPPEVAVFEPSEAEISHTQKATLVCLATGFYPDHVELSWWVNGKEVHSGVSTDPQPLKEQPALNDSRYCLSSRLRVSATFWQNPRNHFRCQVQFYGLSENDEWTQDRAKPVTQIVSAEAWGRADCGFTSESYQQGVLSATILYEILLGKATLYAVLVSALVLMAMVKRKDSRG

SEQ ID NO: 93 - protein, 274 aa, synthetic construct
  REGION 1..274: note = PRAME clone DSK3QLL
MMKSLRVLLVILWLQLSWVWSQQKEVEQNSGPLSVPEGAIASLNCTYSDRGSQSFFWYRQYSGKSPELIMFIYSNGDKEDGRFTAQLNKASQYVSLLIRDSQPSDSATYLCAVKDNAGNMLTFGGGTRLMVKPHIQNPDPAVYQLRDSKSSDKSVCLFTDFDSQTNVSQSKDSDVYITDKTVLDMRSMDFKSNSAVAWSNKSDFACANAFNNSIIPEDTFFPSPESSCDVKLVEKSFETDTNLNFQNLSVIGFRILLLKVAGFNLLMTLRLWSS

SEQ ID NO: 94 - protein, 311 aa, synthetic construct
  REGION 1..311: note = PRAME clone DSK3QLL
MGFRLLCCVAFCLLGAGPVDSGVTQTPKHLITATGQRVTLRCSPRSGDLSVYWYQQSLDQGLQFLIQYYNGEERAKGNILERFSAQQFPDLHSELNLSSLELGDSALYFCASSDGGGVYEQYFGPGTRLTVTEDLKNVFPPEVAVFEPSEAEISHTQKATLVCLATGFYPDHVELSWWVNGKEVHSGVSTDPQPLKEQPALNDSRYCLSSRLRVSATFWQNPRNHFRCQVQFYGLSENDEWTQDRAKPVTQIVSAEAWGRADCGFTSESYQQGVLSATILYEILLGKATLYAVLVSALVLMAMVKRKDSRG

SEQ ID NO: 95 - protein, 6 aa, synthetic construct
  REGION 1..6: note = linker
SGGGSG

SEQ ID NO: 96 - protein, 16 aa, Homo sapiens
MGSNKSKPKDASQRRR

SEQ ID NO: 97 - protein, 5 aa, synthetic construct
  REGION 1..5: note = dual acylation region sequence motif
  VARIANT 4: note = X is any amino acid per ST25 sequence listing standard
MGCXC

SEQ ID NO: 98 - DNA, 19 bp, synthetic construct
  source 1..19: mol_type = other DNA
  misc_feature 1..19: note = PRAME primer sense
cgtttgtggggttccattc

SEQ ID NO: 99 - DNA, 17 bp, synthetic construct
  source 1..17: mol_type = other DNA
  misc_feature 1..17: note = PRAME primer anti-sense
gctccctgggcagcaac

SEQ ID NO: 100 - DNA, 25 bp, synthetic construct
  source 1..25: mol_type = other DNA
  misc_feature 1..25: note = PRAME anti-sense probe
cctgccagctccacaagtctccgtg

SEQ ID NO: 101 - protein, 9 aa, synthetic construct
  REGION 1..9: note = TAA peptide
VLDGLDVLL

SEQ ID NO: 102 - protein, 10 aa, synthetic construct
  REGION 1..10: note = TAA peptide
SLYSFPEPEA

SEQ ID NO: 103 - protein, 10 aa, synthetic construct
  REGION 1..10: note = TAA peptide
ALYVDSLFFL

SEQ ID NO: 104 - protein, 9 aa, synthetic construct
  REGION 1..9: note = TAA peptide
SLLQHLIGL

SEQ ID NO: 105 - protein, 9 aa, synthetic construct
  REGION 1..9: note = TAA peptide
RMFPNAPYL

SEQ ID NO: 106 - protein, 9 aa, synthetic construct
  REGION 1..9: note = TAA peptide
VLQELNVTV

SEQ ID NO: 107 - protein, 9 aa, synthetic construct
  REGION 1..9: note = PRAME epitope
SLLQHLIGL

SEQ ID NO: 108 - protein, 9 aa, synthetic construct
  REGION 1..9: note = PRAME epitope
QLLALLPSL